European Patent Specification EP 4 347 790 B1, published October 22, 2025. Title: Engineering new metabolic pathways in isolated cells for the degradation of guanidinoacetic acid and simultaneous production of creatine. Applicant: EryDel S.p.A. The sequence listing filed with the application follows.

SEQUENCE LISTING (32 sequences)

SEQ ID NO: 1 - protein, 235 aa, Homo sapiens
  SEQ ID NO 1 – Ammino acid sequence of GAMT wild-type without the initial methionine
SAPSATPIFAPGENCSPAWGAAPAAYDAADTHLRILGKPVMERWETPYMHALAAAASSKGGRVLEVGFGMAIAASKVQEAPIDEHWIIECNDGVFQRLRDWAPRQTHKVIPLKGLWEDVAPTLPDGHFDGILYDTYPLSEETWHTHQFNFIKNHAFRLLKPGGVLTYCNLTSWGELMKSKYSDITIMFEETQVPALLEAGFRRENIRTEVMALVPPADCRYYAFPQMITPLVTKG

SEQ ID NO: 2 - protein, 235 aa, Artificial Sequence
  SEQ ID NO 2 – Ammino acid sequence of GAMT CL 32 (A26N-L37M-I187Q-V215Q)
SAPSATPIFAPGENCSPAWGAAPANYDAADTHLRIMGKPVMERWETPYMHALAAAASSKGGRVLEVGFGMAIAASKVQEAPIDEHWIIECNDGVFQRLRDWAPRQTHKVIPLKGLWEDVAPTLPDGHFDGILYDTYPLSEETWHTHQFNFIKNHAFRLLKPGGVLTYCNLTSWGELMKSKYSDITQMFEETQVPALLEAGFRRENIRTEVMALQPPADCRYYAFPQMITPLVTKG

SEQ ID NO: 3 - protein, 235 aa, Artificial Sequence
  SEQ ID NO 3 – Ammino acid sequence of GAMT CL 51 (L37M-I187Q-V215Q)
SAPSATPIFAPGENCSPAWGAAPAAYDAADTHLRIMGKPVMERWETPYMHALAAAASSKGGRVLEVGFGMAIAASKVQEAPIDEHWIIECNDGVFQRLRDWAPRQTHKVIPLKGLWEDVAPTLPDGHFDGILYDTYPLSEETWHTHQFNFIKNHAFRLLKPGGVLTYCNLTSWGELMKSKYSDITQMFEETQVPALLEAGFRRENIRTEVMALQPPADCRYYAFPQMITPLVTKG

SEQ ID NO: 4 - protein, 235 aa, Artificial Sequence
  SEQ ID NO 4 – Ammino acid sequence of GAMT CL 76 (A26N-L37I-I187Q-V215Q)
SAPSATPIFAPGENCSPAWGAAPANYDAADTHLRIIGKPVMERWETPYMHALAAAASSKGGRVLEVGFGMAIAASKVQEAPIDEHWIIECNDGVFQRLRDWAPRQTHKVIPLKGLWEDVAPTLPDGHFDGILYDTYPLSEETWHTHQFNFIKNHAFRLLKPGGVLTYCNLTSWGELMKSKYSDITQMFEETQVPALLEAGFRRENIRTEVMALQPPADCRYYAFPQMITPLVTKG

SEQ ID NO: 5 - protein, 395 aa, Artificial Sequence
  SEQ ID NO 5 – Ammino acid sequence of MAT2A
MNGQLNGFHEAFIEEGTFLFTSESVGEGHPDKICDQISDAVLDAHLQQDPDAKVACETVAKTGMILLAGEITSRAAVDYQKVVREAVKHIGYDDSSKGFDYKTCNVLVALEQQSPDIAQGVHLDRNEEDIGAGDQGLMFGYATDETEECMPLTIVLAHKLNAKLAELRRNGTLPWLRPDSKTQVTVQYMQDRGAVLPIRVHTIVISVQHDEEVCLDEMRDALKEKVIKAVVPAKYLDEDTIYHLQPSGRFVIGGPQGDAGLTGRKIIVDTYGGWGAHGGGAFSGKDYTKVDRSAAYAARWVAKSLVKGGLCRRVLVQVSYAIGVSHPLSISIFHYGTSQKSERELLEIVKKNFDLRPGVIVRDLDLKKPIYQRTAAYGHFGRDSFPWEVPKKLKY

SEQ ID NO: 6 - DNA, 963 bp, Artificial Sequence
  SEQ ID NO 6 – Nucleotidic sequence of His-UB-GAMT wild-type
atggcacatcaccaccaccatcacgtgatgcagatcttcgtgaagaccctgactggtaagaccatcactctcgaggtggagccgagtgacaccattgagaatgtcaaggcaaagatccaagacaaggaaggcatccctcctgaccagcagaggttgatctttgctgggaaacagctggaagatggacgcaccctgtctgactacaacatccagaaagagtccaccctgcacctggtgctccgtctccgcggtggatcggcccccagcgcgacccccatcttcgcgcccggcgagaactgcagccccgcgtggggggcggcgcccgcggcctacgacgcagcggacacgcacctgcgcatcctgggcaagccggtgatggagcgctgggagaccccctatatgcacgcgctggccgccgccgcctcctccaaagggggccgggtcctggaggtgggctttggcatggccatcgcagcgtcaaaggtgcaggaggcgcccattgatgagcattggatcatcgagtgcaatgacggcgtcttccagcggctccgggactgggccccacggcagacacacaaggtcatccccttgaaaggcctgtgggaggatgtggcacccaccctgcctgacggtcactttgatgggatcctgtacgacacgtacccactctcggaggagacctggcacacacaccagttcaacttcatcaagaaccacgcctttcgcctgctgaagccggggggcgtcctcacctactgcaacctcacctcctggggggagctgatgaagtccaagtactcagacatcaccatcatgtttgaggagacgcaggtgcccgcgctgctggaggccggcttccggagggagaacatccgtacggaggtgatggcgctggtcccaccggccgactgccgctactacgccttcccacagatgatcacgcccctggtgaccaaaggctga

SEQ ID NO: 7 - DNA, 963 bp, Artificial Sequence
  SEQ ID NO 7 – Nucleotidic sequence of His-UB-GAMT mutant CLONE 32 (A26N-L37M-I187Q-V215Q)
atggcacatcaccaccaccatcacgtgatgcagatcttcgtgaagaccctgactggtaagaccatcactctcgaggtggagccgagtgacaccattgagaatgtcaaggcaaagatccaagacaaggaaggcatccctcctgaccagcagaggttgatctttgctgggaaacagctggaagatggacgcaccctgtctgactacaacatccagaaagagtccaccctgcacctggtgctccgtctccgcggtggatcggcccccagcgcgacccccatcttcgcgcccggcgagaactgcagccccgcgtggggggcggcgcccgcgaactacgacgcagcggacacgcacctgcgcatcatgggcaagccggtgatggagcgctgggagaccccctatatgcacgcgctggccgccgccgcctcctccaaagggggccgggtcctggaggtgggctttggcatggccatcgcagcgtcaaaggtgcaggaggcgcccattgatgagcattggatcatcgagtgcaatgacggcgtcttccagcggctccgggactgggccccacggcagacacacaaggtcatccccttgaaaggcctgtgggaggatgtggcacccaccctgcctgacggtcactttgatgggatcctgtacgacacgtacccactctcggaggagacctggcacacacaccagttcaacttcatcaagaaccacgcctttcgcctgctgaagccggggggcgtcctcacctactgcaacctcacctcctggggggagctgatgaagtccaagtactcagacatcacccagatgtttgaggagacgcaggtgcccgcgctgctggaggccggcttccggagggagaacatccgtacggaggtgatggcgctgcagccaccggccgactgccgctactacgccttcccacagatgatcacgcccctggtgaccaaaggctga

SEQ ID NO: 8 - DNA, 963 bp, Artificial Sequence
  SEQ ID NO 8 – Nucleotidic sequence of His-UB-GAMT mutant CLONE 51 (L37M-I187Q-V215Q)
atggcacatcaccaccaccatcacgtgatgcagatcttcgtgaagaccctgactggtaagaccatcactctcgaggtggagccgagtgacaccattgagaatgtcaaggcaaagatccaagacaaggaaggcatccctcctgaccagcagaggttgatctttgctgggaaacagctggaagatggacgcaccctgtctgactacaacatccagaaagagtccaccctgcacctggtgctccgtctccgcggtggatcggcccccagcgcgacccccatcttcgcgcccggcgagaactgcagccccgcgtggggggcggcgcccgcggcctacgacgcagcggacacgcacctgcgcatcatgggcaagccggtgatggagcgctgggagaccccctatatgcacgcgctggccgccgccgcctcctccaaagggggccgggtcctggaggtgggctttggcatggccatcgcagcgtcaaaggtgcaggaggcgcccattgatgagcattggatcatcgagtgcaatgacggcgtcttccagcggctccgggactgggccccacggcagacacacaaggtcatccccttgaaaggcctgtgggaggatgtggcacccaccctgcctgacggtcactttgatgggatcctgtacgacacgtacccactctcggaggagacctggcacacacaccagttcaacttcatcaagaaccacgcctttcgcctgctgaagccggggggcgtcctcacctactgcaacctcacctcctggggggagctgatgaagtccaagtactcagacatcacccagatgtttgaggagacgcaggtgcccgcgctgctggaggccggcttccggagggagaacatccgtacggaggtgatggcgctgcagccaccggccgactgccgctactacgccttcccacagatgatcacgcccctggtgaccaaaggctga

SEQ ID NO: 9 - DNA, 963 bp, Artificial Sequence
  SEQ ID NO 9 – Nucleotidic sequence of His-UB-GAMT mutant CLONE 76 (A26N-L37I-I187Q-V215Q)
atggcacatcaccaccaccatcacgtgatgcagatcttcgtgaagaccctgactggtaagaccatcactctcgaggtggagccgagtgacaccattgagaatgtcaaggcaaagatccaagacaaggaaggcatccctcctgaccagcagaggttgatctttgctgggaaacagctggaagatggacgcaccctgtctgactacaacatccagaaagagtccaccctgcacctggtgctccgtctccgcggtggatcggcccccagcgcgacccccatcttcgcgcccggcgagaactgcagccccgcgtggggggcggcgcccgcgaactacgacgcagcggacacgcacctgcgcatcattggcaagccggtgatggagcgctgggagaccccctatatgcacgcgctggccgccgccgcctcctccaaagggggccgggtcctggaggtgggctttggcatggccatcgcagcgtcaaaggtgcaggaggcgcccattgatgagcattggatcatcgagtgcaatgacggcgtcttccagcggctccgggactgggccccacggcagacacacaaggtcatccccttgaaaggcctgtgggaggatgtggcacccaccctgcctgacggtcactttgatgggatcctgtacgacacgtacccactctcggaggagacctggcacacacaccagttcaacttcatcaagaaccacgcctttcgcctgctgaagccggggggcgtcctcacctactgcaacctcacctcctggggggagctgatgaagtccaagtactcagacatcacccagatgtttgaggagacgcaggtgcccgcgctgctggaggccggcttccggagggagaacatccgtacggaggtgatggcgctgcagccaccggccgactgccgctactacgccttcccacagatgatcacgcccctggtgaccaaaggctga

SEQ ID NO: 10 - DNA, 1188 bp, Artificial Sequence
  SEQ ID NO 10 – Nucleotidic sequence of MAT2A wild-type
atgaacggacagctcaacggcttccacgaggcgttcatcgaggagggcacattccttttcacctcagagtcggtcggggaaggccacccagataagatttgtgaccaaatcagtgatgctgtccttgatgcccaccttcagcaggatcctgatgccaaagtagcttgtgaaactgttgctaaaactggaatgatccttcttgctggggaaattacatccagagctgctgttgactaccagaaagtggttcgtgaagctgttaaacacattggatatgatgattcttccaaaggttttgactacaagacttgtaacgtgctggtagccttggagcaacagtcaccagatattgctcaaggtgttcatcttgacagaaatgaagaagacattggtgctggagaccagggcttaatgtttggctatgccactgatgaaactgaggagtgtatgcctttaaccattgtcttggcacacaagctaaatgccaaactggcagaactacgccgtaatggcactttgccttggttacgccctgattctaaaactcaagttactgtgcagtatatgcaggatcgaggtgctgtgcttcccatcagagtccacacaattgttatatctgttcagcatgatgaagaggtttgtcttgatgaaatgagggatgccctaaaggagaaagtcatcaaagcagttgtgcctgcgaaataccttgatgaggatacaatctaccacctacagccaagtggcagatttgttattggtgggcctcagggtgatgctggtttgactggacggaaaatcattgtggacacttatggcggttggggtgctcatggaggaggtgccttttcaggaaaggattataccaaggtcgaccgttcagctgcttatgctgctcgttgggtggcaaaatcccttgttaaaggaggtctgtgccggagggttcttgttcaggtctcttatgctattggagtttctcatccattatctatctccattttccattatggtacctctcagaagagtgagagagagctattagagattgtgaagaagaatttcgatctccgccctggggtcattgtcagggatctggatctgaagaagccaatttatcagaggactgcagcctatggccactttggtagggacagcttcccatgggaagtgcccaaaaagcttaaatattga

SEQ ID NO: 11 - DNA, 1443 bp, Artificial Sequence
  SEQ ID NO 11 – Nucleotidic sequence of His-UB-MAT2A
atggcacatcaccaccaccatcacgtgatgcagatcttcgtgaagaccctgactggtaagaccatcactctcgaggtggagccgagtgacaccattgagaatgtcaaggcaaagatccaagacaaggaaggcatccctcctgaccagcagaggttgatctttgctgggaaacagctggaagatggacgcaccctgtctgactacaacatccagaaagagtccaccctgcacctggtgctccgtctccgcggtggaatgaacggacagctcaacggcttccacgaggcgttcatcgaggagggcacattccttttcacctcagagtcggtcggggaaggccacccagataagatttgtgaccaaatcagtgatgctgtccttgatgcccaccttcagcaggatcctgatgccaaagtagcttgtgaaactgttgctaaaactggaatgatccttcttgctggggaaattacatccagagctgctgttgactaccagaaagtggttcgtgaagctgttaaacacattggatatgatgattcttccaaaggttttgactacaagacttgtaacgtgctggtagccttggagcaacagtcaccagatattgctcaaggtgttcatcttgacagaaatgaagaagacattggtgctggagaccagggcttaatgtttggctatgccactgatgaaactgaggagtgtatgcctttaaccattgtcttggcacacaagctaaatgccaaactggcagaactacgccgtaatggcactttgccttggttacgccctgattctaaaactcaagttactgtgcagtatatgcaggatcgaggtgctgtgcttcccatcagagtccacacaattgttatatctgttcagcatgatgaagaggtttgtcttgatgaaatgagggatgccctaaaggagaaagtcatcaaagcagttgtgcctgcgaaataccttgatgaggatacaatctaccacctacagccaagtggcagatttgttattggtgggcctcagggtgatgctggtttgactggacggaaaatcattgtggacacttatggcggttggggtgctcatggaggaggtgccttttcaggaaaggattataccaaggtcgaccgttcagctgcttatgctgctcgttgggtggcaaaatcccttgttaaaggaggtctgtgccggagggttcttgttcaggtctcttatgctattggagtttctcatccattatctatctccattttccattatggtacctctcagaagagtgagagagagctattagagattgtgaagaagaatttcgatctccgccctggggtcattgtcagggatctggatctgaagaagccaatttatcagaggactgcagcctatggccactttggtagggacagcttcccatgggaagtgcccaaaaagcttaaatattga

SEQ ID NO: 12 - DNA, 34 bp, Artificial Sequence
  SEQ ID NO 12 – GAMT PmlI_Fwd cloning primer
acggtacttcacgtgatgagcgcccccagcgcga

SEQ ID NO: 13 - DNA, 33 bp, Artificial Sequence
  SEQ ID NO 13 - UB-GAMT NcoI_Fwd cloning primer
acggtacttccatgggcccccagcgcgaccccc

SEQ ID NO: 14 - DNA, 37 bp, Artificial Sequence
  SEQ ID NO 14 - GAMT HindIII_Rev cloning primer
ggatacctaaagcttcagcctttggtcaccaggggcg

SEQ ID NO: 15 - DNA, 35 bp, Artificial Sequence
  SEQ ID NO 15 - UB-GAMT (L37I) mutagenesis primer
cacgcacctgcgcatcattggcaagccggtgatgg

SEQ ID NO: 16 - DNA, 33 bp, Artificial Sequence
  SEQ ID NO 16 - UB-GAMT (G38A) mutagenesis primer
acctgcgcatcctggccaagccggtgatggagc

SEQ ID NO: 17 - DNA, 38 bp, Artificial Sequence
  SEQ ID NO 17 - UB-GAMT (L37I - G38A) mutagenesis primer
cacgcacctgcgcatcattgccaagccggtgatggagc

SEQ ID NO: 18 - DNA, 34 bp, Artificial Sequence
  SEQ ID NO 18 - UB-GAMT (L37M) mutagenesis primer
acgcacctgcgcatcatgggcaagccggtgatgg

SEQ ID NO: 19 - DNA, 40 bp, Artificial Sequence
  SEQ ID NO 19 - UB-GAMT (I187Q) mutagenesis primer
gtactcagacatcacccagatgtttgaggagacgcaggtg

SEQ ID NO: 20 - DNA, 32 bp, Artificial Sequence
  SEQ ID NO 20 - UB-GAMT (A26N) mutagenesis primer
gggcggcgcccgcgaactacgacgcagcggac

SEQ ID NO: 21 - DNA, 35 bp, Artificial Sequence
  SEQ ID NO 21 - UB-GAMT (V215Q) mutagenesis primer
ggaggtgatggcgctgcagccaccggccgactgcc

SEQ ID NO: 22 - DNA, 22 bp, Artificial Sequence
  SEQ ID NO 22 - GAMT 7*_Fwd sequencing primer
gcccccagcgcgacccccatct

SEQ ID NO: 23 - DNA, 23 bp, Artificial Sequence
  SEQ ID NO 23 - GAMT 312*_Fwd sequencing primer
acggcagacacacaaggtcatcc

SEQ ID NO: 24 - DNA, 22 bp, Artificial Sequence
  SEQ ID NO 24 - GAMT 711*_Rev sequencing primer
tcagcctttggtcaccaggggc

SEQ ID NO: 25 - DNA, 20 bp, Artificial Sequence
  SEQ ID NO 25 - T7 promoter sequencing primer
taatacgactcactataggg

SEQ ID NO: 26 - DNA, 19 bp, Artificial Sequence
  SEQ ID NO 26 - T7 terminator sequencing primer
gctagttattgctcagcgg

SEQ ID NO: 27 - DNA, 36 bp, Artificial Sequence
  SEQ ID NO 27 - MAT2A SacII_Fwd cloning primer
cgtctccgcggtggaatgaacggacagctcaacggc

SEQ ID NO: 28 - DNA, 42 bp, Artificial Sequence
  SEQ ID NO 28 - MAT2A NotI_Rev cloning primer
cgtctgcggccgctcaatatttaagctttttgggcacttccc

SEQ ID NO: 29 - DNA, 24 bp, Artificial Sequence
  SEQ ID NO 29 - MAT2A 100*_Fwd sequencing primer
gtgaccaaatcagtgatgctgtcc

SEQ ID NO: 30 - DNA, 22 bp, Artificial Sequence
  SEQ ID NO 30 - MAT2A 398*_Fwd sequencing primer
agaccagggcttaatgtttggc

SEQ ID NO: 31 - DNA, 22 bp, Artificial Sequence
  SEQ ID NO 31 - MAT2A 799*_Fwd sequencing primer
ttgtggacacttatggcggttg

SEQ ID NO: 32 - protein, 236 aa, Homo sapiens
  SEQ ID NO 32 – Ammino acid sequence of GAMT wild-type containing the starting methionine
MSAPSATPIFAPGENCSPAWGAAPAAYDAADTHLRILGKPVMERWETPYMHALAAAASSKGGRVLEVGFGMAIAASKVQEAPIDEHWIIECNDGVFQRLRDWAPRQTHKVIPLKGLWEDVAPTLPDGHFDGILYDTYPLSEETWHTHQFNFIKNHAFRLLKPGGVLTYCNLTSWGELMKSKYSDITIMFEETQVPALLEAGFRRENIRTEVMALVPPADCRYYAFPQMITPLVTKG